European Patent Application EP 4 596 574 A1, published August 6, 2025. Title: GLP-1/GCG/GIP三受体激动剂及其用途. Applicant: 广东东阳光药业股份有限公司. Application CN. The sequence listing filed with the application follows.

SEQUENCE LISTING (84 sequences)

SEQ ID NO: 1 - protein, 31 aa, synthetic construct
HAEGTFTSDVSSYLEGQAAKEFIAWLVKGRG

SEQ ID NO: 2 - protein, 29 aa, synthetic construct
HSQGTFTSDYSKYLDSRRAQDFVQWLMNT

SEQ ID NO: 3 - protein, 42 aa, synthetic construct
YAEGTFISDYSIAMDKIHQQDFVNWLLAQKGKKNDWKHNITQ

SEQ ID NO: 4 - protein, 39 aa, synthetic construct
  VARIANT 6: note = X is (L)-alpha-Me-(2-F)-Phe
  VARIANT 2: note = B is Aib
  MOD_RES 17: note = lysine modified by -OEG-gammaGlu-CO-(CH2)18-COOH
YBQGTXTSDYSILLDEKAQRDFIEWLLEGGPSSGAPPPS

SEQ ID NO: 5 - protein, 39 aa, synthetic construct
  VARIANT 2: note = B is Aib
  VARIANT 6: note = X is (L)-alpha-Me-(2-F)-Phe
  MOD_RES 17: note = lysine modified by -OEG-gammaGlu-CO-(CH2)18-COOH
YBHGTXTSDYSILLDEKAQRDFIEWLLAGGPSSGAPPPS

SEQ ID NO: 6 - protein, 39 aa, synthetic construct
  VARIANT 2: note = B is Aib
  VARIANT 6: note = X is (L)-alpha-Me-(2-F)-Phe
  MOD_RES 20: note = lysine modified by -OEG-OEG-gammaGlu-CO-(CH2)18-COOH
YBHGTXTSDYSILLDEIAQKDFIEWLLEGGPSSGAPPPS

SEQ ID NO: 7 - protein, 39 aa, synthetic construct
  VARIANT 2: note = B is Aib
  VARIANT 6: note = X is (L)-alpha-Me-(2-F)-Phe
  MOD_RES 20: note = lysine modified by -OEG-OEG-gammaGlu-CO-(CH2)18-COOH
HBQGTXTSDYSILLDEIAQKDFIEWLLEGGPSSGAPPPS

SEQ ID NO: 8 - protein, 39 aa, synthetic construct
  VARIANT 2: note = B is Aib
  VARIANT 6: note = X is (L)-alpha-Me-(2-F)-Phe
  MOD_RES 17: note = lysine modified by -OEG-gammaGlu-CO-(CH2)18-COOH
YBQGTXTSDYSILLDEKAQQAFIEYLLEGGPSSGAPPPS

SEQ ID NO: 9 - protein, 39 aa, synthetic construct
  VARIANT 2: note = B is Aib
  VARIANT 6: note = X is (L)-alpha-Me-(2-F)-Phe
  MOD_RES 17: note = lysine modified by -OEG-gammaGlu-CO-(CH2)18-COOH
YBQGTXTSDYSILLDEKAQQDFIEWLIAGGPSSGAPPPS

SEQ ID NO: 10 - protein, 39 aa, synthetic construct
  VARIANT 2: note = B is Aib
  VARIANT 6: note = X is (L)-alpha-Me-(2-F)-Phe
  MOD_RES 20: note = lysine modified by -OEG-OEG-gammaGlu-CO-(CH2)18-COOH
YBQGTXTSDYSILLDERAAKEFIEWLLEGGPSSGAPPPS

SEQ ID NO: 11 - protein, 39 aa, synthetic construct
  VARIANT 2: note = B is Aib
  VARIANT 6: note = X is (L)-alpha-Me-(2-F)-Phe
  MOD_RES 20: note = lysine modified by -OEG-OEG-gammaGlu-CO-(CH2)18-COOH
YBQGTXTSDYSILLDERAAKEFIEWLIAGGPSSGAPPPS

SEQ ID NO: 12 - protein, 39 aa, synthetic construct
  VARIANT 2: note = B is Aib
  VARIANT 6: note = X is (L)-alpha-Me-(2-F)-Phe
  MOD_RES 17: note = lysine modified by -OEG-gammaGlu-CO-(CH2)16-COOH
YBHGTXTSDYSILLDEKAQREFIEWLLAGGPSSGAPPPS

SEQ ID NO: 13 - protein, 39 aa, synthetic construct
  VARIANT 2: note = B is Aib
  VARIANT 6: note = X is (L)-alpha-Me-(2-F)-Phe
  MOD_RES 17: note = lysine modified by -OEG-gammaGlu-CO-(CH2)16-COOH
YBHGTXTSDYSILLDEKAQRAFIEYLLAGGPSSGAPPPS

SEQ ID NO: 14 - protein, 39 aa, synthetic construct
  VARIANT 2: note = B is Aib
  VARIANT 6: note = X is (L)-alpha-Me-(2-F)-Phe
  MOD_RES 17: note = lysine modified by -OEG-gammaGlu-CO-(CH2)16-COOH
YBHGTXTSDYSILLDEKAQREFIEWLLEGGPSSGAPPPS

SEQ ID NO: 15 - protein, 39 aa, synthetic construct
  VARIANT 2: note = B is Aib
  VARIANT 6: note = X is (L)-alpha-Me-(2-F)-Phe
  MOD_RES 17: note = lysine modified by -OEG-gammaGlu-CO-(CH2)16-COOH
YBHGTXTSDYSILLDEKRQREFIEWLLAGGPSSGAPPPS

SEQ ID NO: 16 - protein, 39 aa, synthetic construct
  VARIANT 2: note = B is Aib
  VARIANT 6: note = X is (L)-alpha-Me-(2-F)-Phe
  MOD_RES 17: note = lysine modified by -OEG-gammaGlu-CO-(CH2)18-COOH
YBQGTXTSDYSILLDEKAQQEFIEWLLEGGPSSGAPPPS

SEQ ID NO: 17 - protein, 39 aa, synthetic construct; identical to SEQ ID NO: 16
  VARIANT 2: note = B is Aib
  VARIANT 6: note = X is (L)-alpha-Me-(2-F)-Phe
  MOD_RES 17: note = lysine modified by -OEG-gammaGlu-CO-(CH2)16-COOH

SEQ ID NO: 18 - protein, 39 aa, synthetic construct
  VARIANT 6: note = X is (L)-alpha-Me-(2-F)-Phe
  VARIANT 2: note = B is Aib
  MOD_RES 17: note = lysine modified by -OEG-gammaGlu-CO-(CH2)16-COOH
YBHGTXTSDYSILLDEKAQQEFIEWLLAGGPSSGAPPPS

SEQ ID NO: 19 - protein, 39 aa, synthetic construct
  VARIANT 2: note = B is Aib
  VARIANT 6: note = X is (L)-alpha-Me-(2-F)-Phe
  MOD_RES 17: note = lysine modified by -OEG-gammaGlu-CO-(CH2)18-COOH
YBHGTXTSDYSILLDEKAQQAFIEYLLAGGPSSGAPPPS

SEQ ID NO: 20 - protein, 39 aa, synthetic construct
  VARIANT 6: note = X is (L)-alpha-Me-(2-F)-Phe
  VARIANT 2: note = B is Aib
  MOD_RES 17: note = lysine modified by -OEG-gammaGlu-CO-(CH2)16-COOH
YBQGTXTSDYSILLDEKRQQAFIEYLLEGGPSSGAPPPS

SEQ ID NO: 21 - protein, 39 aa, synthetic construct; identical to SEQ ID NO: 13
  VARIANT 2: note = B is Aib
  VARIANT 6: note = X is (L)-alpha-Me-(2-F)-Phe
  MOD_RES 17: note = lysine modified by -OEG-gammaGlu-CO-(CH2)18-COOH

SEQ ID NO: 22 - protein, 39 aa, synthetic construct
  VARIANT 6: note = X is (L)-alpha-Me-(2-F)-Phe
  VARIANT 2: note = B is Aib
  MOD_RES 17: note = lysine modified by -OEG-gammaGlu-CO-(CH2)18-COOH
YBHGTXTSDYSILLDEKAQRAFIEYLLEGGPSSGAPPPS

SEQ ID NO: 23 - protein, 39 aa, synthetic construct
  VARIANT 2: note = B is Aib
  VARIANT 6: note = X is (L)-alpha-Me-(2-F)-Phe
  MOD_RES 17: note = lysine modified by -OEG-gammaGlu-CO-(CH2)18-COOH
YBQGTXTSDYSILLDEKAQRAFIEYLLEGGPSSGAPPPS

SEQ ID NO: 24 - protein, 39 aa, synthetic construct
  VARIANT 6: note = X is (L)-alpha-Me-(2-F)-Phe
  VARIANT 2: note = B is Aib
  MOD_RES 17: note = lysine modified by -OEG-gammaGlu-CO-(CH2)18-COOH
YBQGTXTSDYSILLDEKRQRAFIEYLLAGGPSSGAPPPS

SEQ ID NO: 25 - protein, 39 aa, synthetic construct
  VARIANT 2: note = B is Aib
  VARIANT 6: note = X is (L)-alpha-Me-(2-F)-Phe
  MOD_RES 17: note = lysine modified by -OEG-gammaGlu-CO-(CH2)18-COOH
YBHGTXTSDYSILLDEKRQREFIEWLLEGGPSSGAPPPS

SEQ ID NO: 26 - protein, 39 aa, synthetic construct
  VARIANT 6: note = X is (L)-alpha-Me-(2-F)-Phe
  VARIANT 2: note = B is Aib
  MOD_RES 17: note = lysine modified by -OEG-gammaGlu-CO-(CH2)18-COOH
YBQGTXTSDYSILLDEKRARAFIEYLLAGGPSSGAPPPS

SEQ ID NO: 27 - protein, 39 aa, synthetic construct
  VARIANT 2: note = B is Aib
  VARIANT 6: note = X is (L)-alpha-Me-(2-F)-Phe
  MOD_RES 17: note = lysine modified by -OEG-gammaGlu-CO-(CH2)18-COOH
YBHGTXTSDYSILLDEKRAREFIEWLLEGGPSSGAPPPS

SEQ ID NO: 28 - protein, 39 aa, synthetic construct
  VARIANT 6: note = X is (L)-alpha-Me-(2-F)-Phe
  VARIANT 2: note = B is Aib
  MOD_RES 17: note = lysine modified by -OEG-gammaGlu-CO-(CH2)18-COOH
YBQGTXTSDYSILLDEKAQQEFIEWLLAGGPSSGAPPPS

SEQ ID NO: 29 - protein, 39 aa, synthetic construct
  VARIANT 2: note = B is Aib
  VARIANT 6: note = X is (L)-alpha-Me-(2-F)-Phe
  MOD_RES 17: note = lysine modified by -OEG-gammaGlu-CO-(CH2)18-COOH
YBQGTXTSDYSILLDEKAQQEFIEWLIAGGPSSGAPPPS

SEQ ID NO: 30 - protein, 39 aa, synthetic construct
  VARIANT 6: note = X is (L)-alpha-Me-(2-F)-Phe
  VARIANT 2: note = B is Aib
  MOD_RES 17: note = lysine modified by -OEG-gammaGlu-CO-(CH2)18-COOH
YBQGTXTSDYSILLDEKAQQAFVQWLIAGGPSSGAPPPS

SEQ ID NO: 31 - protein, 39 aa, synthetic construct
  VARIANT 2: note = B is Aib
  VARIANT 6: note = X is (L)-alpha-Me-(2-F)-Phe
  MOD_RES 17: note = lysine modified by -OEG-gammaGlu-CO-(CH2)18-COOH
YBHGTXTSDYSILLDEKRQQAFIEYLLEGGPSSGAPPPS

SEQ ID NO: 32 - protein, 39 aa, synthetic construct
  VARIANT 6: note = X is (L)-alpha-Me-(2-F)-Phe
  VARIANT 2: note = B is Aib
  MOD_RES 17: note = lysine modified by -OEG-gammaGlu-CO-(CH2)18-COOH
YBQGTXTSDYSILLDEKRAQAFIEYLLEGGPSSGAPPPS

SEQ ID NO: 33 - protein, 39 aa, synthetic construct
  VARIANT 2: note = B is Aib
  VARIANT 6: note = X is (L)-alpha-Me-(2-F)-Phe
  MOD_RES 17: note = lysine modified by -OEG-gammaGlu-CO-(CH2)18-COOH
YBQGTXTSDYSILLDEKAQRAFIEYLLAGGPSSGAPPPS

SEQ ID NO: 34 - protein, 39 aa, synthetic construct; identical to SEQ ID NO: 15
  VARIANT 6: note = X is (L)-alpha-Me-(2-F)-Phe
  VARIANT 2: note = B is Aib
  MOD_RES 17: note = lysine modified by -OEG-gammaGlu-CO-(CH2)18-COOH

SEQ ID NO: 35 - protein, 39 aa, synthetic construct
  VARIANT 2: note = B is Aib
  VARIANT 6: note = X is (L)-alpha-Me-(2-F)-Phe
  MOD_RES 17: note = lysine modified by -OEG-gammaGlu-CO-(CH2)18-COOH
YBQGTXTSDYSILLDEKRQRAFIEYLLEGGPSSGAPPPS

SEQ ID NO: 36 - protein, 39 aa, synthetic construct
  VARIANT 6: note = X is (L)-alpha-Me-(2-F)-Phe
  VARIANT 2: note = B is Aib
  MOD_RES 20: note = lysine modified by -OEG-OEG-gammaGlu-CO-(CH2)18-COOH
YBQGTXTSDYSILLDEIAQKAFIEYLLAGGPSSGAPPPS

SEQ ID NO: 37 - protein, 39 aa, synthetic construct
  VARIANT 2: note = B is Aib
  VARIANT 6: note = X is (L)-alpha-Me-(2-F)-Phe
  MOD_RES 20: note = lysine modified by -OEG-OEG-gammaGlu-CO-(CH2)18-COOH
YBQGTXTSDYSILLDEIAQKAFIEYLIAGGPSSGAPPPS

SEQ ID NO: 38 - protein, 39 aa, synthetic construct
  VARIANT 6: note = X is (L)-alpha-Me-(2-F)-Phe
  VARIANT 2: note = 2
  MOD_RES 20: note = lysine modified by -OEG-OEG-gammaGlu-CO-(CH2)18-COOH
YBQGTXTSDYSILLDEIAQKAFVQWLIAGGPSSGAPPPS

SEQ ID NO: 39 - protein, 39 aa, synthetic construct
  VARIANT 6: note = X is (L)-alpha-Me-(2-F)-Phe
  VARIANT 2: note = B is Aib
  MOD_RES 39: note = C-terminal amidation of serine
  MOD_RES 17: note = lysine modified by -OEG-gammaGlu-CO-(CH2)16-COOH
YBHGTXTSDYSILLDEKAQBEFIEWLLAGGPSSGAPPPS

SEQ ID NO: 40 - protein, 39 aa, synthetic construct
  VARIANT 2: note = B is Aib
  VARIANT 6: note = X is (L)-alpha-Me-(2-F)-Phe
  MOD_RES 39: note = C-terminal amidation of serine
  MOD_RES 17: note = lysine modified by -OEG-gammaGlu-CO-(CH2)16-COOH
YBQGTXTSDYSILLDEKAQBAFIEYLLAGGPSSGAPPPS

SEQ ID NO: 41 - protein, 39 aa, synthetic construct
  MOD_RES 39: note = C-terminal amidation of serine
  VARIANT 2: note = B is Aib
  UNSURE 6: note = X is (L)-alpha-Me-(2-F)-Phe
  MOD_RES 17: note = lysine modified by -OEG-gammaGlu-CO-(CH2)16-COOH
YBHGTXTSDYSILLDEKRQBEFIEWLLAGGPSSGAPPPS

SEQ ID NO: 42 - protein, 39 aa, synthetic construct
  MOD_RES 39: note = C-terminal amidation of serine
  VARIANT 2: note = B is Aib
  VARIANT 6: note = X is (L)-alpha-Me-(2-F)-Phe
  METAL 17: note = lysine modified by -OEG-gammaGlu-CO-(CH2)16-COOH
YBQGTXTSDYSILLDEKRQBEFIEWLLAGGPSSGAPPPS

SEQ ID NO: 43 - protein, 39 aa, synthetic construct
  VARIANT 6: note = X is (L)-alpha-Me-(2-F)-Phe
  VARIANT 2: note = B is Aib
  MOD_RES 39: note = C-terminal amidation of serine
  MOD_RES 17: note = lysine modified by -OEG-gammaGlu-CO-(CH2)16-COOH
YBQGTXTSDYSILLDEKRQBAFIEYLLAGGPSSGAPPPS

SEQ ID NO: 44 - protein, 39 aa, synthetic construct
  MOD_RES 39: note = C-terminal amidation of serine
  VARIANT 2: note = B is Aib
  VARIANT 6: note = X is (L)-alpha-Me-(2-F)-Phe
  MOD_RES 14: note = lysine modified by -OEG-gammaGlu-CO-(CH2)16-COOH
YBQGTXTSDYSILKDKIAQQAFIEYLLEGGPSSGAPPPS

SEQ ID NO: 45 - protein, 39 aa, synthetic construct
  VARIANT 6: note = X is (L)-alpha-Me-(2-F)-Phe
  VARIANT 2: note = B is Aib
  MOD_RES 39: note = C-terminal amidation of serine
  MOD_RES 14: note = lysine modified by -OEG-gammaGlu-CO-(CH2)16-COOH
YBQGTXTSDYSILKDKIAQBAFIEYLLEGGPSSGAPPPS

SEQ ID NO: 46 - protein, 39 aa, synthetic construct; identical to SEQ ID NO: 31
  VARIANT 2: note = B is Aib
  VARIANT 6: note = X is (L)-alpha-Me-(2-F)-Phe
  MOD_RES 17: note = lysine modified by -OEG-gammaGlu-CO-(CH2)16-COOH

SEQ ID NO: 47 - protein, 39 aa, synthetic construct
  VARIANT 6: note = X is (L)-alpha-Me-(2-F)-Phe
  VARIANT 2: note = B is Aib
  MOD_RES 17: note = lysine modified by -OEG-gammaGlu-CO-(CH2)16-COOH
YBHGTXTSDYSILLDEKRQRAFIEYLLAGGPSSGAPPPS

SEQ ID NO: 48 - protein, 39 aa, synthetic construct
  VARIANT 2: note = B is Aib
  VARIANT 6: note = X is (L)-alpha-Me-(2-F)-Phe
  MOD_RES 17: note = lysine modified by -OEG-gammaGlu-CO-(CH2)16-COOH
YBHGTXTSDYSILLDEKRQRAFIEYLLEGGPSSGAPPPS

SEQ ID NO: 49 - protein, 39 aa, synthetic construct
  MOD_RES 39: note = C-terminal amidation of serine
  VARIANT 2: note = B is Aib
  VARIANT 6: note = X is (L)-alpha-Me-(2-F)-Phe
  MOD_RES 17: note = lysine modified by -OEG-gammaGlu-CO-(CH2)16-COOH
YBHGTXTSDYSILLDEKRQKAFIEYLLAGGPSSGAPPPS

SEQ ID NO: 50 - protein, 39 aa, synthetic construct
  VARIANT 6: note = X is (L)-alpha-Me-(2-F)-Phe
  VARIANT 2: note = B is Aib
  MOD_RES 14: note = lysine modified by -OEG-gammaGlu-CO-(CH2)16-COOH
  MOD_RES 39: note = C-terminal amidation of serine
YBQGTXTSDYSILKDKIAQQAFIEYLLAGGPSSGAPPPS

SEQ ID NO: 51 - protein, 39 aa, synthetic construct; identical to SEQ ID NO: 35
  VARIANT 2: note = B is Aib
  VARIANT 6: note = X is (L)-alpha-Me-(2-F)-Phe
  MOD_RES 17: note = lysine modified by -OEG-gammaGlu-CO-(CH2)16-COOH

SEQ ID NO: 52 - protein, 39 aa, synthetic construct
  VARIANT 6: note = X is (L)-alpha-Me-(2-F)-Phe
  VARIANT 2: note = B is Aib
  MOD_RES 20: note = lysine modified by -OEG-gammaGlu-CO-(CH2)16-COOH
YBQGTXTSDYSILLDRIRQKEFIEWLLAGGPSSGAPPPS

SEQ ID NO: 53 - protein, 39 aa, synthetic construct
  VARIANT 2: note = B is Aib
  VARIANT 6: note = X is (L)-alpha-Me-(2-F)-Phe
  MOD_RES 20: note = lysine modified by -OEG-gammaGlu-CO-(CH2)16-COOH
YBQGTXTSDYSILLDRIRQKAFIEYLLEGGPSSGAPPPS

SEQ ID NO: 54 - protein, 39 aa, synthetic construct
  VARIANT 6: note = X is (L)-alpha-Me-(2-F)-Phe
  VARIANT 2: note = B is Aib
  MOD_RES 17: note = lysine modified by -OEG-gammaGlu-CO-(CH2)18-COOH
YBQGTXTSDYSILLDRKRQQEFIEWLLAGGPSSGAPPPS

SEQ ID NO: 55 - protein, 39 aa, synthetic construct
  VARIANT 2: note = B is Aib
  VARIANT 6: note = X is (L)-alpha-Me-(2-F)-Phe
  MOD_RES 17: note = lysine modified by -OEG-gammaGlu-CO-(CH2)18-COOH
YBQGTXTSDYSILLDRKRQQAFIEYLLAGGPSSGAPPPS

SEQ ID NO: 56 - protein, 39 aa, synthetic construct
  VARIANT 6: note = X is (L)-alpha-Me-(2-F)-Phe
  VARIANT 2: note = B is Aib
  MOD_RES 39: note = C-terminal amidation of serine
  METAL 17: note = lysine modified by -OEG-gammaGlu-CO-(CH2)16-COOH
YBQGTXTSDYSILLDEKKQBEFIEWLLAGGPSSGAPPPS

SEQ ID NO: 57 - protein, 39 aa, synthetic construct
  MOD_RES 39: note = C-terminal amidation of serine
  VARIANT 2: note = B is Aib
  VARIANT 6: note = X is (L)-alpha-Me-(2-F)-Phe
  MOD_RES 17: note = lysine modified by -OEG-gammaGlu-CO-(CH2)16-COOH
YBQGTXTSDYSILLDEKKQKAFIEYLLAGGPSSGAPPPS

SEQ ID NO: 58 - protein, 39 aa, synthetic construct; identical to SEQ ID NO: 57
  VARIANT 6: note = X is (L)-alpha-Me-(2-F)-Phe
  VARIANT 2: note = B is Aib
  MOD_RES 39: note = C-terminal amidation of serine
  MOD_RES 17: note = lysine modified by -OEG-gammaGlu-CO-(CH2)18-COOH

SEQ ID NO: 59 - protein, 39 aa, synthetic construct; identical to SEQ ID NO: 57
  MOD_RES 39: note = C-terminal amidation of serine
  VARIANT 2: note = B is Aib
  VARIANT 6: note = X is (L)-alpha-Me-(2-F)-Phe
  MOD_RES 20: note = lysine modified by -OEG-gammaGlu-CO-(CH2)16-COOH

SEQ ID NO: 60 - protein, 39 aa, synthetic construct
  VARIANT 6: note = X is (L)-alpha-Me-(2-F)-Phe
  VARIANT 2: note = B is Aib
  MOD_RES 17: note = lysine modified by -OEG-gammaGlu-CO-(CH2)18-COOH
HBQGTXTSDYSILLDEKRQRAFIEYLLAGGPSSGAPPPS

SEQ ID NO: 61 - protein, 39 aa, synthetic construct; identical to SEQ ID NO: 24
  VARIANT 2: note = B is Aib
  VARIANT 6: note = X is (L)-alpha-Me-(2-F)-Phe
  MOD_RES 17: note = lysine modified by -OEG-gammaGlu-CO-(CH2)16-COOH

SEQ ID NO: 62 - protein, 39 aa, synthetic construct
  VARIANT 6: note = X is (L)-alpha-Me-(2-F)-Phe
  VARIANT 2: note = B is Aib
  METAL 17: note = lysine modified by -OEG-gammaGlu-CO-(CH2)16-COOH
YBQGTXTSDYSILLDEKRQRAFVEYLLAGGPSSGAPPPS

SEQ ID NO: 63 - protein, 39 aa, synthetic construct
  VARIANT 2: note = B is Aib
  VARIANT 6: note = X is (L)-alpha-Me-(2-F)-Phe
  MOD_RES 17: note = lysine modified by -OEG-gammaGlu-CO-(CH2)16-COOH
YBQGTXTSDYSIYLDEKAQRAFIEYLLAGGPSSGAPPPS

SEQ ID NO: 64 - protein, 39 aa, synthetic construct
  VARIANT 6: note = X is (L)-alpha-Me-(2-F)-Phe
  VARIANT 2: note = B is Aib
  MOD_RES 17: note = lysine modified by -OEG-gammaGlu-CO-(CH2)16-COOH
YBQGTXTSDYSIYLDEKAQRAFIEYLLEGGPSSGAPPPS

SEQ ID NO: 65 - protein, 39 aa, synthetic construct
  VARIANT 2: note = B is Aib
  VARIANT 6: note = X is (L)-alpha-Me-(2-F)-Phe
  MOD_RES 39: note = C-terminal amidation of serine
  MOD_RES 14: note = lysine modified by -OEG-gammaGlu-CO-(CH2)18-COOH
YBQGTXTSDYSILKDKIAQBAFIEYLLAGGPSSGAPPPS

SEQ ID NO: 66 - protein, 39 aa, synthetic construct; identical to SEQ ID NO: 65
  MOD_RES 39: note = C-terminal amidation of serine
  VARIANT 2: note = B is Aib
  VARIANT 6: note = X is (L)-alpha-Me-(2-F)-Phe
  MOD_RES 14: note = lysine modified by -OEG-gammaGlu-CO-(CH2)16-COOH

SEQ ID NO: 67 - protein, 39 aa, synthetic construct
  VARIANT 6: note = X is (L)-alpha-Me-(2-F)-Phe
  VARIANT 2: note = B is Aib
  MOD_RES 39: note = C-terminal amidation of serine
  MOD_RES 14: note = lysine modified by -OEG-gammaGlu-CO-(CH2)16-COOH
YBQGTXTSDYSILKDKIAQKAFIEYLLAGGPSSGAPPPS

SEQ ID NO: 68 - protein, 39 aa, synthetic construct
  MOD_RES 39: note = C-terminal amidation of serine
  VARIANT 2: note = B is Aib
  VARIANT 6: note = X is (L)-alpha-Me-(2-F)-Phe
  MOD_RES 14: note = lysine modified by -OEG-gammaGlu-CO-(CH2)16-COOH
YBQGTXTSDYSILKDKIAQKAFIEYLLEGGPSSGAPPPS

SEQ ID NO: 69 - protein, 39 aa, synthetic construct
  VARIANT 6: note = X is (L)-alpha-Me-(2-F)-Phe
  VARIANT 2: note = B is Aib
  MOD_RES 14: note = lysine modified by -OEG-gammaGlu-CO-(CH2)16-COOH
YBQGTXTSDYSILKDRIAQRAFIEYLLEGGPSSGAPPPS

SEQ ID NO: 70 - protein, 39 aa, synthetic construct
  VARIANT 2: note = B is Aib
  VARIANT 6: note = X is (L)-alpha-Me-(2-F)-Phe
  MOD_RES 39: note = C-terminal amidation of serine
  MOD_RES 14: note = lysine modified by -OEG-gammaGlu-CO-(CH2)16-COOH
YBQGTXTSDYSILKDKIRQQAFIEYLLEGGPSSGAPPPS

SEQ ID NO: 71 - protein, 39 aa, synthetic construct
  MOD_RES 39: note = C-terminal amidation of serine
  VARIANT 2: note = B is Aib
  VARIANT 6: note = X is (L)-alpha-Me-(2-F)-Phe
  MOD_RES 14: note = lysine modified by -OEG-gammaGlu-CO-(CH2)16-COOH
YBQGTXTSDYSILKDKIRQBAFIEYLLEGGPSSGAPPPS

SEQ ID NO: 72 - protein, 39 aa, synthetic construct
  VARIANT 6: note = X is (L)-alpha-Me-(2-F)-Phe
  MOD_RES 39: note = C-terminal amidation of serine
  VARIANT 2: note = B is Aib
  MOD_RES 14: note = lysine modified by -OEG-gammaGlu-CO-(CH2)16-COOH
YBQGTXTSDYSILKDKIRQBAFIEYLLAGGPSSGAPPPS

SEQ ID NO: 73 - protein, 39 aa, synthetic construct
  VARIANT 2: note = B is Aib
  VARIANT 6: note = X is (L)-alpha-Me-(2-F)-Phe
  MOD_RES 14: note = lysine modified by -OEG-gammaGlu-CO-(CH2)16-COOH
YBQGTXTSDYSILKDRIRQQAFIEYLLEGGPSSGAPPPS

SEQ ID NO: 74 - protein, 39 aa, synthetic construct
  VARIANT 6: note = X is (L)-alpha-Me-(2-F)-Phe
  VARIANT 2: note = B is Aib
  MOD_RES 14: note = lysine modified by -OEG-gammaGlu-CO-(CH2)16-COOH
YBQGTXTSDYSILKDRIRQQAFIEYLLAGGPSSGAPPPS

SEQ ID NO: 75 - protein, 39 aa, synthetic construct
  VARIANT 2: note = B is Aib
  VARIANT 6: note = X is (L)-alpha-Me-(2-F)-Phe
  METAL 14: note = lysine modified by -OEG-gammaGlu-CO-(CH2)16-COOH
YBQGTXTSDYSILKDRRAQQAFVEYLLAGGPSSGAPPPS

SEQ ID NO: 76 - protein, 39 aa, synthetic construct
  VARIANT 6: note = X is (L)-alpha-Me-(2-F)-Phe
  VARIANT 2: note = B is Aib
  MOD_RES 14: note = lysine modified by -OEG-gammaGlu-CO-(CH2)16-COOH
YBQGTXTSDYSILKDRRAQQAFVEYLLEGGPSSGAPPPS

SEQ ID NO: 77 - protein, 39 aa, synthetic construct
  VARIANT 2: note = B is Aib
  VARIANT 6: note = X is (L)-alpha-Me-(2-F)-Phe
  MOD_RES 17: note = lysine modified by -OEG-gammaGlu-CO-(CH2)16-COOH
HBQGTXTSDYSILLDEKRQQAFIEYLLEGGPSSGAPPPS

SEQ ID NO: 78 - protein, 39 aa, synthetic construct
  VARIANT 6: note = X is (L)-alpha-Me-(2-F)-Phe
  VARIANT 2: note = B is Aib
  LIPID 17: note = lysine modified by -OEG-gammaGlu-CO-(CH2)16-COOH
HBQGTXTSDYSILLDEKRQQAFIEYLLAGGPSSGAPPPS

SEQ ID NO: 79 - protein, 39 aa, synthetic construct
  VARIANT 2: note = B is Aib
  VARIANT 6: note = X is (L)-alpha-Me-(2-F)-Phe
  MOD_RES 17: note = lysine modified by -OEG-gammaGlu-CO-(CH2)16-COOH
HBHGTXTSDYSILLDRKAQHAFIEYLLEGGPSSGAPPPS

SEQ ID NO: 80 - protein, 39 aa, synthetic construct
  VARIANT 6: note = X is (L)-alpha-Me-(2-F)-Phe
  VARIANT 2: note = B is Aib
  METAL 17: note = lysine modified by -OEG-gammaGlu-CO-(CH2)16-COOH
HBHGTXTSDYSILLDRKAQQAFIEYLLAGGPSSGAPPPS

SEQ ID NO: 81 - protein, 39 aa, synthetic construct
  VARIANT 2: note = B is Aib
  VARIANT 6: note = X is (L)-alpha-Me-(2-F)-Phe
  MOD_RES 17: note = lysine modified by -OEG-gammaGlu-CO-(CH2)18-COOH
HBHGTXTSDYSILLDRKAQHAFIEYLLAGGPSSGAPPPS

SEQ ID NO: 82 - protein, 39 aa, synthetic construct
  VARIANT 6: note = X is (L)-alpha-Me-(2-F)-Phe
  VARIANT 2: note = B is Aib
  MOD_RES 17: note = lysine modified by -OEG-gammaGlu-CO-(CH2)16-COOH
HBQGTXTSDYSILLDRKAQHAFIEYLLAGGPSSGAPPPS

SEQ ID NO: 83 - protein, 39 aa, synthetic construct
  VARIANT 2: note = B is Aib
  VARIANT 6: note = X is (L)-alpha-Me-(2-F)-Phe
  MOD_RES 17: note = lysine modified by -OEG-gammaGlu-CO-(CH2)18-COOH
HBQGTXTSDYSILLDRKAQHEFIEWLLEGGPSSGAPPPS

SEQ ID NO: 84 - protein, 39 aa, synthetic construct
  VARIANT 6: note = X is (L)-alpha-Me-(2-F)-Phe
  VARIANT 2: note = B is Aib
  METAL 20: note = lysine modified by -OEG-OEG-gammaGlu-CO-(CH2)18-COOH
YBEGTFTSDYSIBLDKIAQKAFVQWLIAGGPSSGAPPPS